European Patent Application EP 4 467 564 A1, published November 27, 2024. Title: ANTIBODY-BOUND LIPID NANOPARTICLE COMPRISING ANTIBODY BOUND TO MEMBRANE SCAFFOLD PROTEIN. Applicant: MVRIX CO.,LTD. The sequence listing filed with the application follows.

SEQUENCE LISTING (30 sequences)

SEQ ID NO: 1 - protein, 525 aa, synthetic construct
MAVQIVESGGGLVQPKESLKISCTASGFTFSNAAIYWVRQTPGKGLEWVGRIRTRPSKYATDYADSVRGRFTISRDDSKSMVYLQMDNLRTEDTAMYYCTPRATEDVPFYWGQGVMVTVSSGGGGSGGGGSGGGGSDIVMTQTPSSQAVSAGEKVTMNCKSSQSVLYDENKKNYLAWYQQKSGQSPKLLIYWASTGESGVPDRFIGSGSGTDFTLTISSVQAEDLAVYYCQQYYDFPPTFGGGTKLELKASGGGGSGGGGSTFSKLREQLGPVTQEFWDNLEKETEGLRQEMSKDLEEVKAKVQPYLDDFQKKWQEEMELYRQKVEPLRAELQEGARQKLHELQEKLSPLGEEMRDRARAHVDALRTHLAPYLDDFQKKWQEEMELYRQKVEPLRAELQEGARQKLHELQEKLSPLGEEMRDRARAHVDALRTHLAPYSDELRQRLAARLEALKENGGARLAEYHAKATEHLSTLSEKAKPALEDLRQGLLPVLESFKVSFLSALEEYTKKLNTQGSGGHHHHHH

SEQ ID NO: 2 - protein, 513 aa, synthetic construct
AVQIVESGGGLVQPKESLKISCTASGFTFSNAAIYWVRQTPGKGLEWVGRIRTRPSKYATDYADSVRGRFTISRDDSKSMVYLQMDNLRTEDTAMYYCTPRATEDVPFYWGQGVMVTVSSGGGGSGGGGSGGGGSDIVMTQTPSSQAVSAGEKVTMNCKSSQSVLYDENKKNYLAWYQQKSGQSPKLLIYWASTGESGVPDRFIGSGSGTDFTLTISSVQAEDLAVYYCQQYYDFPPTFGGGTKLELKASGGGGSGGGGSDEPPQSPWDRVKDLATVYVDVLKDSGRDYVSQFEGSALGKQLNLKLLDNWDSVTSTFSKLREQLGPVTQEFWDNLEKETEGLRQEMSKDLEEVKAKVQPYLDDFQKKWQEEMELYRQKVEPLRAELQEGARQKLHELQEKLSPLGEEMRDRARAHVDALRTHLAPYSDELRQRLAARLEALKENGGARLAEYHAKATEHLSTLSEKAKPALEDLRQGLLPVLESFKVSFLSALEEYTKKLNTQGSGGHHHHHH

SEQ ID NO: 3 - protein, 569 aa, synthetic construct
AVQIVESGGGLVQPKESLKISCTASGFTFSNAAIYWVRQTPGKGLEWVGRIRTRPSKYATDYADSVRGRFTISRDDSKSMVYLQMDNLRTEDTAMYYCTPRATEDVPFYWGQGVMVTVSSGGGGSGGGGSGGGGSDIVMTQTPSSQAVSAGEKVTMNCKSSQSVLYDENKKNYLAWYQQKSGQSPKLLIYWASTGESGVPDRFIGSGSGTDFTLTISSVQAEDLAVYYCQQYYDFPPTFGGGTKLELKASGGGGSGGGGSKVEQAVETEPEPELRQQTEWQSGQRWELALGRFWDYLRWVQTLSEQVQEELLSSQVTQELRALMDETMKELKAYKSELEEQLTPVAEETRARLSKELQAAQARLGADMEDVCGRLVQYRGEVQAMLGQSTEELRVRLASHLRKLRKRLLRDADDLQKRLAVYQAGAREGAERGLSAIRERLGPLVEQGRVRAATVGSLAGQPLQERAQAWGERLRARMEEMGSRTRDRLDEVKEQVAEVRAKLEEQAQQIRLQAEAFQARLKSWFEPLVEDMQRQWAGLVEKVQAAVGTSAAPVPSDNHGSGGHHHHHH

SEQ ID NO: 4 - protein, 523 aa, synthetic construct
MQVQLVESGGGLVQPGGSLRLSCAASGFTFNDFYMNWIRQPPGQAPEWLGVIRNKGNGYTTEVNTSVKGRFTISRDNTQNILYLQMNSLRAEDTAIYYCARGGPYYYSGDDAPYWGQGVMVTVSSGGGGSGGGGSGGGGSDIELTQSPSFLSTSLGNSITITCHASQNIKGWLAWYQQKSGNAPQLLIYKASSLQSGVPSRFSGSGSGTDYIFTISNLQPEDIATYYCQHYQSFPWTFGGGTKLELKASGGGGSGGGGSTFSKLREQLGPVTQEFWDNLEKETEGLRQEMSKDLEEVKAKVQPYLDDFQKKWQEEMELYRQKVEPLRAELQEGARQKLHELQEKLSPLGEEMRDRARAHVDALRTHLAPYLDDFQKKWQEEMELYRQKVEPLRAELQEGARQKLHELQEKLSPLGEEMRDRARAHVDALRTHLAPYSDELRQRLAARLEALKENGGARLAEYHAKATEHLSTLSEKAKPALEDLRQGLLPVLESFKVSFLSALEEYTKKLNTQGSGGHHHHHH

SEQ ID NO: 5 - protein, 512 aa, synthetic construct
MQVQLVESGGGLVQPGGSLRLSCAASGFTFNDFYMNWIRQPPGQAPEWLGVIRNKGNGYTTEVNTSVKGRFTISRDNTQNILYLQMNSLRAEDTAIYYCARGGPYYYSGDDAPYWGQGVMVTVSSGGGGSGGGGSGGGGSDIELTQSPSFLSTSLGNSITITCHASQNIKGWLAWYQQKSGNAPQLLIYKASSLQSGVPSRFSGSGSGTDYIFTISNLQPEDIATYYCQHYQSFPWTFGGGTKLELKASGGGGSGGGGSDEPPQSPWDRVKDLATVYVDVLKDSGRDYVSQFEGSALGKQLNLKLLDNWDSVTSTFSKLREQLGPVTQEFWDNLEKETEGLRQEMSKDLEEVKAKVQPYLDDFQKKWQEEMELYRQKVEPLRAELQEGARQKLHELQEKLSPLGEEMRDRARAHVDALRTHLAPYSDELRQRLAARLEALKENGGARLAEYHAKATEHLSTLSEKAKPALEDLRQGLLPVLESFKVSFLSALEEYTKKLNTQGSGGHHHHHH

SEQ ID NO: 6 - protein, 568 aa, synthetic construct
MQVQLVESGGGLVQPGGSLRLSCAASGFTFNDFYMNWIRQPPGQAPEWLGVIRNKGNGYTTEVNTSVKGRFTISRDNTQNILYLQMNSLRAEDTAIYYCARGGPYYYSGDDAPYWGQGVMVTVSSGGGGSGGGGSGGGGSDIELTQSPSFLSTSLGNSITITCHASQNIKGWLAWYQQKSGNAPQLLIYKASSLQSGVPSRFSGSGSGTDYIFTISNLQPEDIATYYCQHYQSFPWTFGGGTKLELKASGGGGSGGGGSKVEQAVETEPEPELRQQTEWQSGQRWELALGRFWDYLRWVQTLSEQVQEELLSSQVTQELRALMDETMKELKAYKSELEEQLTPVAEETRARLSKELQAAQARLGADMEDVCGRLVQYRGEVQAMLGQSTEELRVRLASHLRKLRKRLLRDADDLQKRLAVYQAGAREGAERGLSAIRERLGPLVEQGRVRAATVGSLAGQPLQERAQAWGERLRARMEEMGSRTRDRLDEVKEQVAEVRAKLEEQAQQIRLQAEAFQARLKSWFEPLVEDMQRQWAGLVEKVQAAVGTSAAPVPSDNHGSGGHHHHHH

SEQ ID NO: 7 - protein, 537 aa, synthetic construct
MAAQPAMADYKQAVVTQESALTTSPGETVTLTCRSSTGAVTISNYANWVQEKPDHLFTGLIGGTNNRAPGVPARFSGSLIGDKAALTITGAQTEDEAIYFCALWYNNQFIFGSGTKVTVLGGGGGSGGGGSGGGGSGGGGSEVQLQQSGPVLVKPGASVKMSCKASGNTFTDSFMHWMKQSHGKSLEWIGIINPYNGGTSYNQKFKGKATLTVDKSSSTAYMELNSLTSEDSAVYYCARNGVRYYFDYWGQGTTLTVSSASGAGGGGSGGGGSTFSKLREQLGPVTQEFWDNLEKETEGLRQEMSKDLEEVKAKVQPYLDDFQKKWQEEMELYRQKVEPLRAELQEGARQKLHELQEKLSPLGEEMRDRARAHVDALRTHLAPYLDDFQKKWQEEMELYRQKVEPLRAELQEGARQKLHELQEKLSPLGEEMRDRARAHVDALRTHLAPYSDELRQRLAARLEALKENGGARLAEYHAKATEHLSTLSEKAKPALEDLRQGLLPVLESFKVSFLSALEEYTKKLNTQGSGGHHHHHH

SEQ ID NO: 8 - protein, 526 aa, synthetic construct
MAAQPAMADYKQAVVTQESALTTSPGETVTLTCRSSTGAVTISNYANWVQEKPDHLFTGLIGGTNNRAPGVPARFSGSLIGDKAALTITGAQTEDEAIYFCALWYNNQFIFGSGTKVTVLGGGGGSGGGGSGGGGSGGGGSEVQLQQSGPVLVKPGASVKMSCKASGNTFTDSFMHWMKQSHGKSLEWIGIINPYNGGTSYNQKFKGKATLTVDKSSSTAYMELNSLTSEDSAVYYCARNGVRYYFDYWGQGTTLTVSSASGAGGGGSGGGGSDEPPQSPWDRVKDLATVYVDVLKDSGRDYVSQFEGSALGKQLNLKLLDNWDSVTSTFSKLREQLGPVTQEFWDNLEKETEGLRQEMSKDLEEVKAKVQPYLDDFQKKWQEEMELYRQKVEPLRAELQEGARQKLHELQEKLSPLGEEMRDRARAHVDALRTHLAPYSDELRQRLAARLEALKENGGARLAEYHAKATEHLSTLSEKAKPALEDLRQGLLPVLESFKVSFLSALEEYTKKLNTQGSGGHHHHHH

SEQ ID NO: 9 - protein, 582 aa, synthetic construct
MAAQPAMADYKQAVVTQESALTTSPGETVTLTCRSSTGAVTISNYANWVQEKPDHLFTGLIGGTNNRAPGVPARFSGSLIGDKAALTITGAQTEDEAIYFCALWYNNQFIFGSGTKVTVLGGGGGSGGGGSGGGGSGGGGSEVQLQQSGPVLVKPGASVKMSCKASGNTFTDSFMHWMKQSHGKSLEWIGIINPYNGGTSYNQKFKGKATLTVDKSSSTAYMELNSLTSEDSAVYYCARNGVRYYFDYWGQGTTLTVSSASGAGGGGSGGGGSKVEQAVETEPEPELRQQTEWQSGQRWELALGRFWDYLRWVQTLSEQVQEELLSSQVTQELRALMDETMKELKAYKSELEEQLTPVAEETRARLSKELQAAQARLGADMEDVCGRLVQYRGEVQAMLGQSTEELRVRLASHLRKLRKRLLRDADDLQKRLAVYQAGAREGAERGLSAIRERLGPLVEQGRVRAATVGSLAGQPLQERAQAWGERLRARMEEMGSRTRDRLDEVKEQVAEVRAKLEEQAQQIRLQAEAFQARLKSWFEPLVEDMQRQWAGLVEKVQAAVGTSAAPVPSDNHGSGGHHHHHH

SEQ ID NO: 10 - protein, 743 aa, synthetic construct
MAVQIVESGGGLVQPKESLKISCTASGFTFSNAAIYWVRQTPGKGLEWVGRIRTRPSKYATDYADSVRGRFTISRDDSKSMVYLQMDNLRTEDTAMYYCTPRATEDVPFYWGQGVMVTVSSGGGGSGGGGSGGGGSDIVMTQTPSSQAVSAGEKVTMNCKSSQSVLYDENKKNYLAWYQQKSGQSPKLLIYWASTGESGVPDRFIGSGSGTDFTLTISSVQAEDLAVYYCQQYYDFPPTFGGGTKLELKLEPKSCDKTHTCPPCPAPELLGGPSVFLFPPKPKDTLMISRTPEVTCVVVDVSHEDPEVKFNWYVDGVEVHNAKTKPREEQYNSTYRVVSVLTVLHQDWLNGKEYKCKVSNKALPAPIEKTISKAKGQPREPQVYTLPPSRDELTKNQVSLTCLVKGFYPSDIAVEWESNGQPENNYKTTPPVLDSDGSFFLYSKLTVDKSRWQQGNVFSCSVMHEALHNHYTQKSLSLSPGKASGGGGSTFSKLREQLGPVTQEFWDNLEKETEGLRQEMSKDLEEVKAKVQPYLDDFQKKWQEEMELYRQKVEPLRAELQEGARQKLHELQEKLSPLGEEMRDRARAHVDALRTHLAPYLDDFQKKWQEEMELYRQKVEPLRAELQEGARQKLHELQEKLSPLGEEMRDRARAHVDALRTHLAPYSDELRQRLAARLEALKENGGARLAEYHAKATEHLSTLSEKAKPALEDLRQGLLPVLESFKVSFLSALEEYTKKLNTQ

SEQ ID NO: 11 - protein, 732 aa, synthetic construct
MAVQIVESGGGLVQPKESLKISCTASGFTFSNAAIYWVRQTPGKGLEWVGRIRTRPSKYATDYADSVRGRFTISRDDSKSMVYLQMDNLRTEDTAMYYCTPRATEDVPFYWGQGVMVTVSSGGGGSGGGGSGGGGSDIVMTQTPSSQAVSAGEKVTMNCKSSQSVLYDENKKNYLAWYQQKSGQSPKLLIYWASTGESGVPDRFIGSGSGTDFTLTISSVQAEDLAVYYCQQYYDFPPTFGGGTKLELKLEPKSCDKTHTCPPCPAPELLGGPSVFLFPPKPKDTLMISRTPEVTCVVVDVSHEDPEVKFNWYVDGVEVHNAKTKPREEQYNSTYRVVSVLTVLHQDWLNGKEYKCKVSNKALPAPIEKTISKAKGQPREPQVYTLPPSRDELTKNQVSLTCLVKGFYPSDIAVEWESNGQPENNYKTTPPVLDSDGSFFLYSKLTVDKSRWQQGNVFSCSVMHEALHNHYTQKSLSLSPGKASGGGGSDEPPQSPWDRVKDLATVYVDVLKDSGRDYVSQFEGSALGKQLNLKLLDNWDSVTSTFSKLREQLGPVTQEFWDNLEKETEGLRQEMSKDLEEVKAKVQPYLDDFQKKWQEEMELYRQKVEPLRAELQEGARQKLHELQEKLSPLGEEMRDRARAHVDALRTHLAPYSDELRQRLAARLEALKENGGARLAEYHAKATEHLSTLSEKAKPALEDLRQGLLPVLESFKVSFLSALEEYTKKLNTQ

SEQ ID NO: 12 - protein, 788 aa, synthetic construct
MAVQIVESGGGLVQPKESLKISCTASGFTFSNAAIYWVRQTPGKGLEWVGRIRTRPSKYATDYADSVRGRFTISRDDSKSMVYLQMDNLRTEDTAMYYCTPRATEDVPFYWGQGVMVTVSSGGGGSGGGGSGGGGSDIVMTQTPSSQAVSAGEKVTMNCKSSQSVLYDENKKNYLAWYQQKSGQSPKLLIYWASTGESGVPDRFIGSGSGTDFTLTISSVQAEDLAVYYCQQYYDFPPTFGGGTKLELKLEPKSCDKTHTCPPCPAPELLGGPSVFLFPPKPKDTLMISRTPEVTCVVVDVSHEDPEVKFNWYVDGVEVHNAKTKPREEQYNSTYRVVSVLTVLHQDWLNGKEYKCKVSNKALPAPIEKTISKAKGQPREPQVYTLPPSRDELTKNQVSLTCLVKGFYPSDIAVEWESNGQPENNYKTTPPVLDSDGSFFLYSKLTVDKSRWQQGNVFSCSVMHEALHNHYTQKSLSLSPGKASGGGGSKVEQAVETEPEPELRQQTEWQSGQRWELALGRFWDYLRWVQTLSEQVQEELLSSQVTQELRALMDETMKELKAYKSELEEQLTPVAEETRARLSKELQAAQARLGADMEDVCGRLVQYRGEVQAMLGQSTEELRVRLASHLRKLRKRLLRDADDLQKRLAVYQAGAREGAERGLSAIRERLGPLVEQGRVRAATVGSLAGQPLQERAQAWGERLRARMEEMGSRTRDRLDEVKEQVAEVRAKLEEQAQQIRLQAEAFQARLKSWFEPLVEDMQRQWAGLVEKVQAAVGTSAAPVPSDNH

SEQ ID NO: 13 - protein, 741 aa, synthetic construct
MQVQLVESGGGLVQPGGSLRLSCAASGFTFNDFYMNWIRQPPGQAPEWLGVIRNKGNGYTTEVNTSVKGRFTISRDNTQNILYLQMNSLRAEDTAIYYCARGGPYYYSGDDAPYWGQGVMVTVSSGGGGSGGGGSGGGGSDIELTQSPSFLSTSLGNSITITCHASQNIKGWLAWYQQKSGNAPQLLIYKASSLQSGVPSRFSGSGSGTDYIFTISNLQPEDIATYYCQHYQSFPWTFGGGTKLELKLEPKSCDKTHTCPPCPAPELLGGPSVFLFPPKPKDTLMISRTPEVTCVVVDVSHEDPEVKFNWYVDGVEVHNAKTKPREEQYNSTYRVVSVLTVLHQDWLNGKEYKCKVSNKALPAPIEKTISKAKGQPREPQVYTLPPSRDELTKNQVSLTCLVKGFYPSDIAVEWESNGQPENNYKTTPPVLDSDGSFFLYSKLTVDKSRWQQGNVFSCSVMHEALHNHYTQKSLSLSPGKASGGGGSTFSKLREQLGPVTQEFWDNLEKETEGLRQEMSKDLEEVKAKVQPYLDDFQKKWQEEMELYRQKVEPLRAELQEGARQKLHELQEKLSPLGEEMRDRARAHVDALRTHLAPYLDDFQKKWQEEMELYRQKVEPLRAELQEGARQKLHELQEKLSPLGEEMRDRARAHVDALRTHLAPYSDELRQRLAARLEALKENGGARLAEYHAKATEHLSTLSEKAKPALEDLRQGLLPVLESFKVSFLSALEEYTKKLNTQ

SEQ ID NO: 14 - protein, 730 aa, synthetic construct
MQVQLVESGGGLVQPGGSLRLSCAASGFTFNDFYMNWIRQPPGQAPEWLGVIRNKGNGYTTEVNTSVKGRFTISRDNTQNILYLQMNSLRAEDTAIYYCARGGPYYYSGDDAPYWGQGVMVTVSSGGGGSGGGGSGGGGSDIELTQSPSFLSTSLGNSITITCHASQNIKGWLAWYQQKSGNAPQLLIYKASSLQSGVPSRFSGSGSGTDYIFTISNLQPEDIATYYCQHYQSFPWTFGGGTKLELKLEPKSCDKTHTCPPCPAPELLGGPSVFLFPPKPKDTLMISRTPEVTCVVVDVSHEDPEVKFNWYVDGVEVHNAKTKPREEQYNSTYRVVSVLTVLHQDWLNGKEYKCKVSNKALPAPIEKTISKAKGQPREPQVYTLPPSRDELTKNQVSLTCLVKGFYPSDIAVEWESNGQPENNYKTTPPVLDSDGSFFLYSKLTVDKSRWQQGNVFSCSVMHEALHNHYTQKSLSLSPGKASGGGGSDEPPQSPWDRVKDLATVYVDVLKDSGRDYVSQFEGSALGKQLNLKLLDNWDSVTSTFSKLREQLGPVTQEFWDNLEKETEGLRQEMSKDLEEVKAKVQPYLDDFQKKWQEEMELYRQKVEPLRAELQEGARQKLHELQEKLSPLGEEMRDRARAHVDALRTHLAPYSDELRQRLAARLEALKENGGARLAEYHAKATEHLSTLSEKAKPALEDLRQGLLPVLESFKVSFLSALEEYTKKLNTQ

SEQ ID NO: 15 - protein, 786 aa, synthetic construct
MQVQLVESGGGLVQPGGSLRLSCAASGFTFNDFYMNWIRQPPGQAPEWLGVIRNKGNGYTTEVNTSVKGRFTISRDNTQNILYLQMNSLRAEDTAIYYCARGGPYYYSGDDAPYWGQGVMVTVSSGGGGSGGGGSGGGGSDIELTQSPSFLSTSLGNSITITCHASQNIKGWLAWYQQKSGNAPQLLIYKASSLQSGVPSRFSGSGSGTDYIFTISNLQPEDIATYYCQHYQSFPWTFGGGTKLELKLEPKSCDKTHTCPPCPAPELLGGPSVFLFPPKPKDTLMISRTPEVTCVVVDVSHEDPEVKFNWYVDGVEVHNAKTKPREEQYNSTYRVVSVLTVLHQDWLNGKEYKCKVSNKALPAPIEKTISKAKGQPREPQVYTLPPSRDELTKNQVSLTCLVKGFYPSDIAVEWESNGQPENNYKTTPPVLDSDGSFFLYSKLTVDKSRWQQGNVFSCSVMHEALHNHYTQKSLSLSPGKASGGGGSKVEQAVETEPEPELRQQTEWQSGQRWELALGRFWDYLRWVQTLSEQVQEELLSSQVTQELRALMDETMKELKAYKSELEEQLTPVAEETRARLSKELQAAQARLGADMEDVCGRLVQYRGEVQAMLGQSTEELRVRLASHLRKLRKRLLRDADDLQKRLAVYQAGAREGAERGLSAIRERLGPLVEQGRVRAATVGSLAGQPLQERAQAWGERLRARMEEMGSRTRDRLDEVKEQVAEVRAKLEEQAQQIRLQAEAFQARLKSWFEPLVEDMQRQWAGLVEKVQAAVGTSAAPVPSDNH

SEQ ID NO: 16 - protein, 757 aa, synthetic construct
MAAQPAMADYKQAVVTQESALTTSPGETVTLTCRSSTGAVTISNYANWVQEKPDHLFTGLIGGTNNRAPGVPARFSGSLIGDKAALTITGAQTEDEAIYFCALWYNNQFIFGSGTKVTVLGGGGGSGGGGSGGGGSGGGGSEVQLQQSGPVLVKPGASVKMSCKASGNTFTDSFMHWMKQSHGKSLEWIGIINPYNGGTSYNQKFKGKATLTVDKSSSTAYMELNSLTSEDSAVYYCARNGVRYYFDYWGQGTTLTVSSASGALEPKSCDKTHTCPPCPAPELLGGPSVFLFPPKPKDTLMISRTPEVTCVVVDVSHEDPEVKFNWYVDGVEVHNAKTKPREEQYNSTYRVVSVLTVLHQDWLNGKEYKCKVSNKALPAPIEKTISKAKGQPREPQVYTLPPSRDELTKNQVSLTCLVKGFYPSDIAVEWESNGQPENNYKTTPPVLDSDGSFFLYSKLTVDKSRWQQGNVFSCSVMHEALHNHYTQKSLSLSPGKASGGGGSTFSKLREQLGPVTQEFWDNLEKETEGLRQEMSKDLEEVKAKVQPYLDDFQKKWQEEMELYRQKVEPLRAELQEGARQKLHELQEKLSPLGEEMRDRARAHVDALRTHLAPYLDDFQKKWQEEMELYRQKVEPLRAELQEGARQKLHELQEKLSPLGEEMRDRARAHVDALRTHLAPYSDELRQRLAARLEALKENGGARLAEYHAKATEHLSTLSEKAKPALEDLRQGLLPVLESFKVSFLSALEEYTKKLNTQ

SEQ ID NO: 17 - protein, 746 aa, synthetic construct
MAAQPAMADYKQAVVTQESALTTSPGETVTLTCRSSTGAVTISNYANWVQEKPDHLFTGLIGGTNNRAPGVPARFSGSLIGDKAALTITGAQTEDEAIYFCALWYNNQFIFGSGTKVTVLGGGGGSGGGGSGGGGSGGGGSEVQLQQSGPVLVKPGASVKMSCKASGNTFTDSFMHWMKQSHGKSLEWIGIINPYNGGTSYNQKFKGKATLTVDKSSSTAYMELNSLTSEDSAVYYCARNGVRYYFDYWGQGTTLTVSSASGALEPKSCDKTHTCPPCPAPELLGGPSVFLFPPKPKDTLMISRTPEVTCVVVDVSHEDPEVKFNWYVDGVEVHNAKTKPREEQYNSTYRVVSVLTVLHQDWLNGKEYKCKVSNKALPAPIEKTISKAKGQPREPQVYTLPPSRDELTKNQVSLTCLVKGFYPSDIAVEWESNGQPENNYKTTPPVLDSDGSFFLYSKLTVDKSRWQQGNVFSCSVMHEALHNHYTQKSLSLSPGKASGGGGSDEPPQSPWDRVKDLATVYVDVLKDSGRDYVSQFEGSALGKQLNLKLLDNWDSVTSTFSKLREQLGPVTQEFWDNLEKETEGLRQEMSKDLEEVKAKVQPYLDDFQKKWQEEMELYRQKVEPLRAELQEGARQKLHELQEKLSPLGEEMRDRARAHVDALRTHLAPYSDELRQRLAARLEALKENGGARLAEYHAKATEHLSTLSEKAKPALEDLRQGLLPVLESFKVSFLSALEEYTKKLNTQ

SEQ ID NO: 18 - protein, 802 aa, synthetic construct
MAAQPAMADYKQAVVTQESALTTSPGETVTLTCRSSTGAVTISNYANWVQEKPDHLFTGLIGGTNNRAPGVPARFSGSLIGDKAALTITGAQTEDEAIYFCALWYNNQFIFGSGTKVTVLGGGGGSGGGGSGGGGSGGGGSEVQLQQSGPVLVKPGASVKMSCKASGNTFTDSFMHWMKQSHGKSLEWIGIINPYNGGTSYNQKFKGKATLTVDKSSSTAYMELNSLTSEDSAVYYCARNGVRYYFDYWGQGTTLTVSSASGALEPKSCDKTHTCPPCPAPELLGGPSVFLFPPKPKDTLMISRTPEVTCVVVDVSHEDPEVKFNWYVDGVEVHNAKTKPREEQYNSTYRVVSVLTVLHQDWLNGKEYKCKVSNKALPAPIEKTISKAKGQPREPQVYTLPPSRDELTKNQVSLTCLVKGFYPSDIAVEWESNGQPENNYKTTPPVLDSDGSFFLYSKLTVDKSRWQQGNVFSCSVMHEALHNHYTQKSLSLSPGKASGGGGSKVEQAVETEPEPELRQQTEWQSGQRWELALGRFWDYLRWVQTLSEQVQEELLSSQVTQELRALMDETMKELKAYKSELEEQLTPVAEETRARLSKELQAAQARLGADMEDVCGRLVQYRGEVQAMLGQSTEELRVRLASHLRKLRKRLLRDADDLQKRLAVYQAGAREGAERGLSAIRERLGPLVEQGRVRAATVGSLAGQPLQERAQAWGERLRARMEEMGSRTRDRLDEVKEQVAEVRAKLEEQAQQIRLQAEAFQARLKSWFEPLVEDMQRQWAGLVEKVQAAVGTSAAPVPSDNH

SEQ ID NO: 19 - protein, 220 aa, synthetic construct
MDIVMTQTPSSQAVSAGEKVTMNCKSSQSVLYDENKKNYLAWYQQKSGQSPKLLIYWASTGESGVPDRFIGSGSGTDFTLTISSVQAEDLAVYYCQQYYDFPPTFGGGTKLELKTVAAPSVFIFPPSDEQLKSGTASVVCLLNNFYPREAKVQWKVDNALQSGNSQESVTEQDSKDSTYSLSSTLTLSKADYEKHKVYACEVTHQGLSSPVTKSFNRGEC

SEQ ID NO: 20 - protein, 214 aa, synthetic construct
MDIELTQSPSFLSTSLGNSITITCHASQNIKGWLAWYQQKSGNAPQLLIYKASSLQSGVPSRFSGSGSGTDYIFTISNLQPEDIATYYCQHYQSFPWTFGGGTKLELKTVAAPSVFIFPPSDEQLKSGTASVVCLLNNFYPREAKVQWKVDNALQSGNSQESVTEQDSKDSTYSLSSTLTLSKADYEKHKVYACEVTHQGLSSPVTKSFNRGEC

SEQ ID NO: 21 - protein, 227 aa, synthetic construct
MAAQPAMADYKQAVVTQESALTTSPGETVTLTCRSSTGAVTISNYANWVQEKPDHLFTGLIGGTNNRAPGVPARFSGSLIGDKAALTITGAQTEDEAIYFCALWYNNQFIFGSGTKVTVLGTVAAPSVFIFPPSDEQLKSGTASVVCLLNNFYPREAKVQWKVDNALQSGNSQESVTEQDSKDSTYSLSSTLTLSKADYEKHKVYACEVTHQGLSSPVTKSFNRGEC

SEQ ID NO: 22 - protein, 711 aa, synthetic construct
MAVQIVESGGGLVQPKESLKISCTASGFTFSNAAIYWVRQTPGKGLEWVGRIRTRPSKYATDYADSVRGRFTISRDDSKSMVYLQMDNLRTEDTAMYYCTPRATEDVPFYWGQGVMVTVSSASTKGPSVFPLAPSSKSTSGGTAALGCLVKDYFPEPVTVSWNSGALTSGVHTFPAVLQSSGLYSLSSVVTVPSSSLGTQTYICNVNHKPSNTKVDKKVEPPKSCDKTHTCPPCPAPELLGGPSVFLFPPKPKDTLMISRTPEVTCVVVDVSHEDPEVKFNWYVDGVEVHNAKTKPREEQYNSTYRVVSVLTVLHQDWLNGKEYKCKVSNKALPAPIEKTISKAKGQPREPQVYTLPPSRDELTKNQVSLTCLVKGFYPSDIAVEWESNGQPENNYKTTPPVLDSDGSFFLYSKLTVDKSRWQQGNVFSCSVMHEALHNHYTQKSLSLSPGKGGGGSTFSKLREQLGPVTQEFWDNLEKETEGLRQEMSKDLEEVKAKVQPYLDDFQKKWQEEMELYRQKVEPLRAELQEGARQKLHELQEKLSPLGEEMRDRARAHVDALRTHLAPYLDDFQKKWQEEMELYRQKVEPLRAELQEGARQKLHELQEKLSPLGEEMRDRARAHVDALRTHLAPYSDELRQRLAARLEALKENGGARLAEYHAKATEHLSTLSEKAKPALEDLRQGLLPVLESFKVSFLSALEEYTKKLNTQ

SEQ ID NO: 23 - protein, 700 aa, synthetic construct
MAVQIVESGGGLVQPKESLKISCTASGFTFSNAAIYWVRQTPGKGLEWVGRIRTRPSKYATDYADSVRGRFTISRDDSKSMVYLQMDNLRTEDTAMYYCTPRATEDVPFYWGQGVMVTVSSASTKGPSVFPLAPSSKSTSGGTAALGCLVKDYFPEPVTVSWNSGALTSGVHTFPAVLQSSGLYSLSSVVTVPSSSLGTQTYICNVNHKPSNTKVDKKVEPPKSCDKTHTCPPCPAPELLGGPSVFLFPPKPKDTLMISRTPEVTCVVVDVSHEDPEVKFNWYVDGVEVHNAKTKPREEQYNSTYRVVSVLTVLHQDWLNGKEYKCKVSNKALPAPIEKTISKAKGQPREPQVYTLPPSRDELTKNQVSLTCLVKGFYPSDIAVEWESNGQPENNYKTTPPVLDSDGSFFLYSKLTVDKSRWQQGNVFSCSVMHEALHNHYTQKSLSLSPGKGGGGSDEPPQSPWDRVKDLATVYVDVLKDSGRDYVSQFEGSALGKQLNLKLLDNWDSVTSTFSKLREQLGPVTQEFWDNLEKETEGLRQEMSKDLEEVKAKVQPYLDDFQKKWQEEMELYRQKVEPLRAELQEGARQKLHELQEKLSPLGEEMRDRARAHVDALRTHLAPYSDELRQRLAARLEALKENGGARLAEYHAKATEHLSTLSEKAKPALEDLRQGLLPVLESFKVSFLSALEEYTKKLNTQ

SEQ ID NO: 24 - protein, 756 aa, synthetic construct
MAVQIVESGGGLVQPKESLKISCTASGFTFSNAAIYWVRQTPGKGLEWVGRIRTRPSKYATDYADSVRGRFTISRDDSKSMVYLQMDNLRTEDTAMYYCTPRATEDVPFYWGQGVMVTVSSASTKGPSVFPLAPSSKSTSGGTAALGCLVKDYFPEPVTVSWNSGALTSGVHTFPAVLQSSGLYSLSSVVTVPSSSLGTQTYICNVNHKPSNTKVDKKVEPPKSCDKTHTCPPCPAPELLGGPSVFLFPPKPKDTLMISRTPEVTCVVVDVSHEDPEVKFNWYVDGVEVHNAKTKPREEQYNSTYRVVSVLTVLHQDWLNGKEYKCKVSNKALPAPIEKTISKAKGQPREPQVYTLPPSRDELTKNQVSLTCLVKGFYPSDIAVEWESNGQPENNYKTTPPVLDSDGSFFLYSKLTVDKSRWQQGNVFSCSVMHEALHNHYTQKSLSLSPGKGGGGSKVEQAVETEPEPELRQQTEWQSGQRWELALGRFWDYLRWVQTLSEQVQEELLSSQVTQELRALMDETMKELKAYKSELEEQLTPVAEETRARLSKELQAAQARLGADMEDVCGRLVQYRGEVQAMLGQSTEELRVRLASHLRKLRKRLLRDADDLQKRLAVYQAGAREGAERGLSAIRERLGPLVEQGRVRAATVGSLAGQPLQERAQAWGERLRARMEEMGSRTRDRLDEVKEQVAEVRAKLEEQAQQIRLQAEAFQARLKSWFEPLVEDMQRQWAGLVEKVQAAVGTSAAPVPSDNH

SEQ ID NO: 25 - protein, 715 aa, synthetic construct
MQVQLVESGGGLVQPGGSLRLSCAASGFTFNDFYMNWIRQPPGQAPEWLGVIRNKGNGYTTEVNTSVKGRFTISRDNTQNILYLQMNSLRAEDTAIYYCARGGPYYYSGDDAPYWGQGVMVTVSSASTKGPSVFPLAPSSKSTSGGTAALGCLVKDYFPEPVTVSWNSGALTSGVHTFPAVLQSSGLYSLSSVVTVPSSSLGTQTYICNVNHKPSNTKVDKKVEPPKSCDKTHTCPPCPAPELLGGPSVFLFPPKPKDTLMISRTPEVTCVVVDVSHEDPEVKFNWYVDGVEVHNAKTKPREEQYNSTYRVVSVLTVLHQDWLNGKEYKCKVSNKALPAPIEKTISKAKGQPREPQVYTLPPSRDELTKNQVSLTCLVKGFYPSDIAVEWESNGQPENNYKTTPPVLDSDGSFFLYSKLTVDKSRWQQGNVFSCSVMHEALHNHYTQKSLSLSPGKGGGGSTFSKLREQLGPVTQEFWDNLEKETEGLRQEMSKDLEEVKAKVQPYLDDFQKKWQEEMELYRQKVEPLRAELQEGARQKLHELQEKLSPLGEEMRDRARAHVDALRTHLAPYLDDFQKKWQEEMELYRQKVEPLRAELQEGARQKLHELQEKLSPLGEEMRDRARAHVDALRTHLAPYSDELRQRLAARLEALKENGGARLAEYHAKATEHLSTLSEKAKPALEDLRQGLLPVLESFKVSFLSALEEYTKKLNTQ

SEQ ID NO: 26 - protein, 704 aa, synthetic construct
MQVQLVESGGGLVQPGGSLRLSCAASGFTFNDFYMNWIRQPPGQAPEWLGVIRNKGNGYTTEVNTSVKGRFTISRDNTQNILYLQMNSLRAEDTAIYYCARGGPYYYSGDDAPYWGQGVMVTVSSASTKGPSVFPLAPSSKSTSGGTAALGCLVKDYFPEPVTVSWNSGALTSGVHTFPAVLQSSGLYSLSSVVTVPSSSLGTQTYICNVNHKPSNTKVDKKVEPPKSCDKTHTCPPCPAPELLGGPSVFLFPPKPKDTLMISRTPEVTCVVVDVSHEDPEVKFNWYVDGVEVHNAKTKPREEQYNSTYRVVSVLTVLHQDWLNGKEYKCKVSNKALPAPIEKTISKAKGQPREPQVYTLPPSRDELTKNQVSLTCLVKGFYPSDIAVEWESNGQPENNYKTTPPVLDSDGSFFLYSKLTVDKSRWQQGNVFSCSVMHEALHNHYTQKSLSLSPGKGGGGSDEPPQSPWDRVKDLATVYVDVLKDSGRDYVSQFEGSALGKQLNLKLLDNWDSVTSTFSKLREQLGPVTQEFWDNLEKETEGLRQEMSKDLEEVKAKVQPYLDDFQKKWQEEMELYRQKVEPLRAELQEGARQKLHELQEKLSPLGEEMRDRARAHVDALRTHLAPYSDELRQRLAARLEALKENGGARLAEYHAKATEHLSTLSEKAKPALEDLRQGLLPVLESFKVSFLSALEEYTKKLNTQ

SEQ ID NO: 27 - protein, 760 aa, synthetic construct
MQVQLVESGGGLVQPGGSLRLSCAASGFTFNDFYMNWIRQPPGQAPEWLGVIRNKGNGYTTEVNTSVKGRFTISRDNTQNILYLQMNSLRAEDTAIYYCARGGPYYYSGDDAPYWGQGVMVTVSSASTKGPSVFPLAPSSKSTSGGTAALGCLVKDYFPEPVTVSWNSGALTSGVHTFPAVLQSSGLYSLSSVVTVPSSSLGTQTYICNVNHKPSNTKVDKKVEPPKSCDKTHTCPPCPAPELLGGPSVFLFPPKPKDTLMISRTPEVTCVVVDVSHEDPEVKFNWYVDGVEVHNAKTKPREEQYNSTYRVVSVLTVLHQDWLNGKEYKCKVSNKALPAPIEKTISKAKGQPREPQVYTLPPSRDELTKNQVSLTCLVKGFYPSDIAVEWESNGQPENNYKTTPPVLDSDGSFFLYSKLTVDKSRWQQGNVFSCSVMHEALHNHYTQKSLSLSPGKGGGGSKVEQAVETEPEPELRQQTEWQSGQRWELALGRFWDYLRWVQTLSEQVQEELLSSQVTQELRALMDETMKELKAYKSELEEQLTPVAEETRARLSKELQAAQARLGADMEDVCGRLVQYRGEVQAMLGQSTEELRVRLASHLRKLRKRLLRDADDLQKRLAVYQAGAREGAERGLSAIRERLGPLVEQGRVRAATVGSLAGQPLQERAQAWGERLRARMEEMGSRTRDRLDEVKEQVAEVRAKLEEQAQQIRLQAEAFQARLKSWFEPLVEDMQRQWAGLVEKVQAAVGTSAAPVPSDNH

SEQ ID NO: 28 - protein, 713 aa, synthetic construct
MEVQLQQSGPVLVKPGASVKMSCKASGNTFTDSFMHWMKQSHGKSLEWIGIINPYNGGTSYNQKFKGKATLTVDKSSSTAYMELNSLTSEDSAVYYCARNGVRYYFDYWGQGTTLTVSSASGAASTKGPSVFPLAPSSKSTSGGTAALGCLVKDYFPEPVTVSWNSGALTSGVHTFPAVLQSSGLYSLSSVVTVPSSSLGTQTYICNVNHKPSNTKVDKKVEPPKSCDKTHTCPPCPAPELLGGPSVFLFPPKPKDTLMISRTPEVTCVVVDVSHEDPEVKFNWYVDGVEVHNAKTKPREEQYNSTYRVVSVLTVLHQDWLNGKEYKCKVSNKALPAPIEKTISKAKGQPREPQVYTLPPSRDELTKNQVSLTCLVKGFYPSDIAVEWESNGQPENNYKTTPPVLDSDGSFFLYSKLTVDKSRWQQGNVFSCSVMHEALHNHYTQKSLSLSPGKGGGGSTFSKLREQLGPVTQEFWDNLEKETEGLRQEMSKDLEEVKAKVQPYLDDFQKKWQEEMELYRQKVEPLRAELQEGARQKLHELQEKLSPLGEEMRDRARAHVDALRTHLAPYLDDFQKKWQEEMELYRQKVEPLRAELQEGARQKLHELQEKLSPLGEEMRDRARAHVDALRTHLAPYSDELRQRLAARLEALKENGGARLAEYHAKATEHLSTLSEKAKPALEDLRQGLLPVLESFKVSFLSALEEYTKKLNTQ

SEQ ID NO: 29 - protein, 702 aa, synthetic construct
MEVQLQQSGPVLVKPGASVKMSCKASGNTFTDSFMHWMKQSHGKSLEWIGIINPYNGGTSYNQKFKGKATLTVDKSSSTAYMELNSLTSEDSAVYYCARNGVRYYFDYWGQGTTLTVSSASGAASTKGPSVFPLAPSSKSTSGGTAALGCLVKDYFPEPVTVSWNSGALTSGVHTFPAVLQSSGLYSLSSVVTVPSSSLGTQTYICNVNHKPSNTKVDKKVEPPKSCDKTHTCPPCPAPELLGGPSVFLFPPKPKDTLMISRTPEVTCVVVDVSHEDPEVKFNWYVDGVEVHNAKTKPREEQYNSTYRVVSVLTVLHQDWLNGKEYKCKVSNKALPAPIEKTISKAKGQPREPQVYTLPPSRDELTKNQVSLTCLVKGFYPSDIAVEWESNGQPENNYKTTPPVLDSDGSFFLYSKLTVDKSRWQQGNVFSCSVMHEALHNHYTQKSLSLSPGKGGGGSDEPPQSPWDRVKDLATVYVDVLKDSGRDYVSQFEGSALGKQLNLKLLDNWDSVTSTFSKLREQLGPVTQEFWDNLEKETEGLRQEMSKDLEEVKAKVQPYLDDFQKKWQEEMELYRQKVEPLRAELQEGARQKLHELQEKLSPLGEEMRDRARAHVDALRTHLAPYSDELRQRLAARLEALKENGGARLAEYHAKATEHLSTLSEKAKPALEDLRQGLLPVLESFKVSFLSALEEYTKKLNTQ

SEQ ID NO: 30 - protein, 758 aa, synthetic construct
MEVQLQQSGPVLVKPGASVKMSCKASGNTFTDSFMHWMKQSHGKSLEWIGIINPYNGGTSYNQKFKGKATLTVDKSSSTAYMELNSLTSEDSAVYYCARNGVRYYFDYWGQGTTLTVSSASGAASTKGPSVFPLAPSSKSTSGGTAALGCLVKDYFPEPVTVSWNSGALTSGVHTFPAVLQSSGLYSLSSVVTVPSSSLGTQTYICNVNHKPSNTKVDKKVEPPKSCDKTHTCPPCPAPELLGGPSVFLFPPKPKDTLMISRTPEVTCVVVDVSHEDPEVKFNWYVDGVEVHNAKTKPREEQYNSTYRVVSVLTVLHQDWLNGKEYKCKVSNKALPAPIEKTISKAKGQPREPQVYTLPPSRDELTKNQVSLTCLVKGFYPSDIAVEWESNGQPENNYKTTPPVLDSDGSFFLYSKLTVDKSRWQQGNVFSCSVMHEALHNHYTQKSLSLSPGKGGGGSKVEQAVETEPEPELRQQTEWQSGQRWELALGRFWDYLRWVQTLSEQVQEELLSSQVTQELRALMDETMKELKAYKSELEEQLTPVAEETRARLSKELQAAQARLGADMEDVCGRLVQYRGEVQAMLGQSTEELRVRLASHLRKLRKRLLRDADDLQKRLAVYQAGAREGAERGLSAIRERLGPLVEQGRVRAATVGSLAGQPLQERAQAWGERLRARMEEMGSRTRDRLDEVKEQVAEVRAKLEEQAQQIRLQAEAFQARLKSWFEPLVEDMQRQWAGLVEKVQAAVGTSAAPVPSDNH